European Patent Application EP 4 442 835 A1, published October 9, 2024. Title: 分析方法. Applicant: DENSO CORPORATION. The sequence listing filed with the application follows.

SEQUENCE LISTING (4 sequences)

SEQ ID NO: 1 - DNA, 51 bp, synthetic construct
  source 1..51: mol_type = other DNA
cagcaccgaccttgtgctttgggagtgctggtccaagggcgttaatggaca

SEQ ID NO: 2 - DNA, 58 bp, synthetic construct
  source 1..58: mol_type = other DNA
gctggatgtcgcttacgacaatattccttaggggcaccgctacattgacacatccagc

SEQ ID NO: 3 - DNA, 51 bp, synthetic construct
  source 1..51: mol_type = other DNA
gatatcaacccatggtaggtattgcttggtagggatagtgggcttgatgtt

SEQ ID NO: 4 - DNA, 58 bp, synthetic construct
  source 1..58: mol_type = other DNA
gctggatgtcaccggattgtcggacatcggattgtctgagtcatatgacacatccagc